European Patent Application EP 4 286 515 A1, published December 6, 2023. Title: C-glycosyltransferase variants and Use thereof. Applicant: Korea Advanced Institute of Science and Technology. The sequence listing filed with the application follows.

SEQUENCE LISTING (122 sequences)

SEQ ID NO: 1 - protein, 477 aa, Gentiana triflora
MGSLTNNDNLHIFLVCFIGQGVVNPMLRLGKAFASKGLLVTLSAPEIVGTEIRKANNLNDDQPIKVGSGMIRFEFFDDGWESVNGSKPFDVWVYINHLDQTGRQKLPIMLKKHEETGTPVSCLILNPLVPWVADVADSLQIPCATLWVQSCASFSAYYHYHHGLVPFPTESEPEIDVQLPGMPLLKYDEVPDYLHPRTPYPFFGTNILGQFKNLSKNFCILMDTFYELEHEIIDNMCKLCPIKPIGPLFKIPKDPSSNGITGNFMKVDDCKEWLDSRPTSTVVYVSVGSVVYLKQEQVTEMAYGILNSEVSFLWVLRPPSKRIGTEPHVLPEEFWEKAGDRGKVVQWSPQEQVLAHPATVGFLTHCGWNSTQEAISSGVPVITFPQFGDQVTNAKFLVEEFKVGVRLGRGELENRIITRDEVERALREITSGPKAEEVKENALKWKKKAEETVAKGGYSERNLVGFIEEVARKTGTK

SEQ ID NO: 2 - protein, 536 aa, Streptomyces peucetius
MALTKPDVDVLVVGGGLGGLSTALFLARRGARVLLVERHASTSVLPKAAGQNPRTMELFRFGGVADEILATDDIRGAQGDFTIKVVERVGGRVLHSFAESFEELVGATEQCTPMPWALAPQDRVEPVLVAHAAKHGAEIRFATELTSFQAGDDGVTARLRDLGTGAESTVSARYLVAADGPRSAIRESLGITRHGHGTLAHFMGVIFEADLTAVVPPGSTGWYYLQHPDFTGTFGPTDRPNRHTFYVRYDPERGERPEDYTPQRCTELIRLAVDAPGLVPDILDIQAWDMAAYIADRWREGPVLLVGDAAKVTPPTGGMGGNTAIGDGFDVAWKLAAVLRGEAGERLLDSYGAERSLVSRLVVDESLAIYAQRMAPHLLGSVPEERGTAQVVLGFRYRSTAVAAEDDDPEPTEDPRRPSGRPGFRAPHVWIEQDGTRRSTVELFGDCWVLLAAPEGGAWGQAAARAAADLGVRLDVHLVGRDVAAPSGELTRTYGIGRAGASLVRPDGVVAWRTAVAPGAEAQDQLSTLLTRLLAR

SEQ ID NO: 3 - DNA, 37 bp, Artificial Sequence
  Primer
aaacactacgtggctagccaaaaaacccctcaagacc

SEQ ID NO: 4 - DNA, 35 bp, Artificial Sequence
  Primer
aaagcatgcactagttaatacgactcactataggg

SEQ ID NO: 5 - DNA, 47 bp, Artificial Sequence
  Primer
ctttaagaaggagatatacatatgataataaataacagaaatgaatc

SEQ ID NO: 6 - DNA, 49 bp, Artificial Sequence
  Primer
cttgtcgacggagctcgaattcattaatttttatcgtttaaacttgatg

SEQ ID NO: 7 - DNA, 61 bp, Artificial Sequence
  Primer
gaattcgagctccgtcgacaaataaggagatataccatggacgatatttctttatcatctg

SEQ ID NO: 8 - DNA, 53 bp, Artificial Sequence
  Primer
gtggtgctcgagtgcggccgcaagcttattactcatctttgttccttataatc

SEQ ID NO: 9 - DNA, 46 bp, Artificial Sequence
  Primer
ctttaagaaggagatatacatatgaaactaatctctatgttgttac

SEQ ID NO: 10 - DNA, 47 bp, Artificial Sequence
  Primer
cttgtcgacggagctcgaattcattattgattcctcaatgtaaatag

SEQ ID NO: 11 - DNA, 45 bp, Artificial Sequence
  Primer
ctttaagaaggagatatacatatgcgtcatgtagagcatacagtc

SEQ ID NO: 12 - DNA, 47 bp, Artificial Sequence
  Primer
cttgtcgacggagctcgaattcttattaatcctcttcctcttgctcg

SEQ ID NO: 13 - DNA, 43 bp, Artificial Sequence
  Primer
ctttaagaaggagatatacatatggccttgacgaagccggatg

SEQ ID NO: 14 - DNA, 41 bp, Artificial Sequence
  Primer
caagcttgtcgacggagctcgagttgtcggagcggctggcc

SEQ ID NO: 15 - DNA, 24 bp, Artificial Sequence
  Primer
ctttaagaaggagatatacatatg

SEQ ID NO: 16 - DNA, 41 bp, Artificial Sequence
  Primer
caaaacagccaagcttgcatgcaagcttgtcgacggagctc

SEQ ID NO: 17 - DNA, 21 bp, Artificial Sequence
  Primer
catgcaagcttggctgttttg

SEQ ID NO: 18 - DNA, 24 bp, Artificial Sequence
  Primer
catatgtatatctccttcttaaag

SEQ ID NO: 19 - DNA, 48 bp, Artificial Sequence
  Primer
gttaagtataagaaggagatatacatatgcgtcgactgcctgatttag

SEQ ID NO: 20 - DNA, 52 bp, Artificial Sequence
  Primer
gatatccaattgagatctgccttatgattaccctttctgtaccattgtgatc

SEQ ID NO: 21 - DNA, 47 bp, Artificial Sequence
  Primer
caatttcacacaggaaacagaattcatggctgccattaatacgaaag

SEQ ID NO: 22 - DNA, 43 bp, Artificial Sequence
  Primer
ccgggtaccgagctcgaattcattacttcttaatgcccatctc

SEQ ID NO: 23 - DNA, 64 bp, Artificial Sequence
  Primer
gtaatgaattcgagctcggtacccaatttcacacaggaaacagaatggcaatccacaatcgtgc

SEQ ID NO: 24 - DNA, 44 bp, Artificial Sequence
  Primer
ctctagaggatccccgggtaccattacgcgtttttcagaacttc

SEQ ID NO: 25 - DNA, 68 bp, Artificial Sequence
  Primer
ctagagtcgacctgcaggcatgccaatttcacacaggaaacagaatggctattgaacgtactttttcc

SEQ ID NO: 26 - DNA, 42 bp, Artificial Sequence
  Primer
caaaacagccaagcttgcatgcattaacgggtgcgcgggcac

SEQ ID NO: 27 - DNA, 30 bp, Artificial Sequence
  Primer
gtcgtaccgaaggggtccaccggctggtac

SEQ ID NO: 28 - DNA, 30 bp, Artificial Sequence
  Primer
ggtggaccccttcggtacgacggcggtgag

SEQ ID NO: 29 - DNA, 30 bp, Artificial Sequence
  Primer
gacgtatggcaatacatcaatcacttagac

SEQ ID NO: 30 - DNA, 30 bp, Artificial Sequence
  Primer
gattgatgtattgccatacgtcaaacggtt

SEQ ID NO: 31 - DNA, 30 bp, Artificial Sequence
  Primer
gtgcccgacttcctgcatccgcgcacaccc

SEQ ID NO: 32 - DNA, 30 bp, Artificial Sequence
  Primer
cggatgcaggaagtcgggcacttcatcata

SEQ ID NO: 33 - DNA, 42 bp, Artificial Sequence
  Primer
ctttaataaggagatataccatggccttgacgaagccggatg

SEQ ID NO: 34 - DNA, 40 bp, Artificial Sequence
  Primer
ccgagctcgaattcggatcccaagcttgtcgacggagctc

SEQ ID NO: 35 - DNA, 42 bp, Artificial Sequence
  Primer
gtataagaaggagatatacatatggcagatgtcctgcaggag

SEQ ID NO: 36 - DNA, 43 bp, Artificial Sequence
  Primer
gatatccaattgagatctgccaattagggaatggggacgctac

SEQ ID NO: 37 - DNA, 261 bp, Unknown
  Streptomyces ravidus
atgtccagtttcagtattgatgatctgaagcgtatcttgcgcgaaggggcaggggcaacggctgagttagacggtgacattttagacgcctcctttgatgatttggggtatgattctttggctcttcttgaaacgggttcgcgcatcggacgtgaatacggtttggaatttgaggatacagctttcgccgacgtggaaacacctcgtgacttggtcggcgtagttaatgctcagttatcggccccggctccgcgtgggtaa

SEQ ID NO: 38 - DNA, 1321 bp, Unknown
  Streptomyces sp. R1128
atgcgtcatgtagagcatacagtcaccgttgcggccccagcagacttggtttgggaggtacttgccgatgtcttaggctatgctgacatcttcccaccgacggaaaaagttgaaattcttgaggaggggcaaggataccaggtagtgcgccttcacgtcgatgttgcgggtgagattaatacatggaccagtcgtcgcgatttagaccctgcgcgccgcgtaattgcttaccgccaacttgagacggctccgatcgtgggccacatgagcggggaatggcgtgctttcacactggatgccgaacgtacccaattagtcctgactcacgatttcgtaacccgtgcagccggggatgacggtttagtcgccggaaaattgaccccagatgaggcgcgcgaaatgttagaagcggtggtagaacgtaactctgtcgccgacttaaacgcggtccttggagaagctgagcgtcgcgtccgcgcagccggtggagttggtaccgtaactgcgtaataataattttgtttaactttaagaaggagatatatccatgtcagggcgcaaaacctttttagacttaagttttgctacccgcgacacaccgtcggaggcgactccggtggtggtagatttgctggaccacgtaactggagccaccgtattaggattatcacctgaggatttccccgatggtatggctatttccaatgagaccgttacgttgacgacccacactggcacgcacatggatgcgccactgcactatggtcccttaagtgggggagttccggcaaagtcgattgaccaagtgcccttggaatggtgctatggacctggagttcgtttggatgttcgccacgtgccggcaggagatggtattactgtcgatcatttgaacgccgcgttggatgcagcagagcacgatttggcccccggtgacattgtgatgctgtggaccggcgcggacgctctgtggggaacccgcgaatacttgagcacgtttccggggttaactgggaaggggacacaatttttggtcgaggcgggtgttaaagtcattggcattgatgcatggggactggatcgcccgatggcagctatgatcgaagaataccgtcgtacgggcgataaaggagcattatggccggctcacgtctatggacgcacacgcgaatacctgcaattagagaagcttaataatttgggcgctttaccaggagctacagggtatgacatttcatgctttccggttgcggttgcaggcactggagctgggtggactcgtgtggtcgccgttttcgagcaagaggaagaggattaataa

SEQ ID NO: 39 - DNA, 1482 bp, Arabidopsis thaliana
atgtcccatcgccgcaaccgtagccacaacaatcgtttacccccgggacctaatccctggcccattatcggaaacctgccgcacatgggtacgaagccccaccgtacgttgtcggctatggttacgacctatggcccaattctgcacctgcgtctgggttttgtagacgtggtcgtagcggcgtccaagtcggtcgccgagcagttcttgaagattcacgacgctaacttcgcttcacgtccccccaactcaggagccaaacacatggcgtataattatcaagacttggtattcgccccctatggacatcgctggcgcttattgcgcaagatcagctcggtgcatctgttctcggcaaaagcgttggaggactttaaacacgtgcgtcaggaagaggtcggaacactgactcgcgaattagtacgtgtcggcaccaaaccagtgaaccttgggcaactggtgaatatgtgcgttgtcaacgccttaggacgcgaaatgatcggacgccgcttattcggggccgatgccgatcataaggcggatgagttccgctcgatggtcacggagatgatggcgttagcgggggtctttaatatcggcgactttgtaccgtcattagactggcttgatctgcaaggggtcgctggaaagatgaagcgtttacataagcgttttgatgcgttcttaagttcgattttaaaagaacatgaaatgaatgggcaagaccaaaagcataccgatatgttatcgaccttaatcagccttaagggtacagatctggatggggatggcggctccttaacggatactgaaattaaggcgcttttattaaacatgttcacagccggaaccgacacatcagccagtacagtagattgggcaatcgctgaattgatccgccaccccgatatcatggtgaaggctcaggaagaattagatattgttgtaggtcgcgaccgccctgtgaatgagtctgatatcgcccaactgccgtacttacaggcggtaattaaggaaaattttcgtctgcatccacctactcccctgtctttgccgcacattgcgagtgaatcctgtgagattaacggttaccatattcccaaaggttcaacattacttaccaacatctgggctatcgcccgtgatccggaccagtggagcgatccgttagcttttaaaccagaacgttttctgccaggaggagaaaaatctggggttgatgtaaaaggtagtgatttcgagctgattccgttcggtgcaggccgtcgcatttgtgcaggcctgtctctgggtcttcgcacgatccagttcttaacagcgactttagtacaagggtttgattgggagttagctgggggagtgacgcccgaaaaactgaacatggaagaatcgtacgggttaactttgcaacgcgctgtccctctggtagtacacccgaaacctcgtttggccccgaatgtgtacgggctgggcagtggctaa

SEQ ID NO: 40 - DNA, 2136 bp, Arabidopsis thaliana
atgtcttcttcttcttcttcttctacctctatgatcgacctgatggctgctatcatcaaaggtgaaccggttatcgtttctgacccggctaacgcttctgcttacgaatctgttgctgctgaactgtcttctatgttaattgagaatcgtcagtttgctatgatcgttacaacatccatcgcggtccttattggttgtatcgttatgttggtctggcgccgctctggttccggtaactctaaacgtgtggaaccgcttaaaccgctggtgatcaaacctcgtgaggaggaaatcgacgatggacgtaaaaaagtaacaatctttttcggaacgcagactggcactgcggaaggttttgccaaggcattaggtgaggaagctaaagctcgttatgaaaagacgcgcttcaagattgttgatctggacgattacgctgcagacgatgatgaatacgaggaaaaattaaaaaaagaggatgtagctttcttcttcttagctacgtatggcgatggtgaaccgacagataatgccgctcgtttttataagtggtttaccgaaggcaatgatcgtggtgagtggttgaaaaacttaaaatatggggttttcgggctgggcaatcgtcaatacgagcactttaacaaggtcgcgaaagtggtcgatgacattctggttgagcaaggcgcacagcgtctggtacaagtagggttaggggatgatgaccagtgtatcgaagatgatttcacagcttggcgcgaagcattgtggcccgagttggatacgattctgcgcgaagagggcgatacggctgttgccacaccctacacagccgcagtattagagtatcgcgtaagcatccatgatagcgaggatgccaaattcaatgatattaaccttgctaacggaaacgggtatacagtttttgacgctcaacatccgtataaggccaacgttgcggtcaaacgtgaattgcacaccccggagtccgaccgttcctgtatccatctggaatttgatattgcgggatcaggtttaacatacgaaactggagatcacgttggtgttctgtgcgataacttatccgagacggtggatgaggcactgcgccttttagacatgtcccctgacacgtattttagcttgcatgctgaaaaagaggacggtactccgatcagtagctcgctgccaccgccgtttccaccgtgcaatttacgcacggctttaacacgttacgcgtgcctgttgtcatctcctaagaaatccgccttagtggctttggctgcacacgctagtgatcccactgaggccgagcgcttgaaacacttagcaagccctgcaggtaaagacgagtactccaagtgggtagtagagtcacagcgtagtttattggaggtgatggccgagtttcctagtgcgaagccaccgttgggagttttctttgccggggtggctccgcgtttgcaaccacgtttttatagcatcagtagttctccaaaaatcgccgagactcgcattcacgttacatgtgccctggtctacgaaaaaatgccgactgggcgcatccacaagggtgtatgctcgacttggatgaagaacgccgtaccctacgaaaagtctgaaaactgcagctcggcgccaatcttcgtacgccagtccaatttcaagttgccgtcagattcaaaggtaccgatcattatgatcggtccaggaacggggttagctccgttccgtgggttcttacaggaacgcttagcactggtcgagtcgggggtagaattgggcccctccgtcttgtttttcgggtgtcgtaaccgtcgcatggacttcatctatgaagaagagctgcaacgtttcgtggaaagtggggcgcttgctgaactgtcggtggcgttttcccgcgaaggacccacgaaagaatatgttcaacacaaaatgatggacaaagcgtcggatatctggaacatgatttcacagggcgcttatttatatgtatgtggcgatgcgaaaggcatggcgcgtgacgtccaccgttctctgcacaccattgcgcaagagcaaggtagcatggattcaacgaaagcagaaggcttcgtgaagaatttacaaacctctgggcgctatcttcgtgatgtgtggtaa

SEQ ID NO: 41 - DNA, 1098 bp, Unknown
  Streptomyces fradiae Tu2717
atgtttgccctggctccgctggccacagcagctcgtaatgcaggtcatcaggtagtaatggcagcaaaccaggacatgggacctgtcgtaaccggggttggccttccagccgtagcaaccactgatcttccgatccgtcatttcatcactaccgatcgtgaaggacgtcccgaggccattccttctgacccggtcgcgcaggcccgtttcactggtcgctggttcgcccgtatggctgccagttccttgccccgtatgcttgatttttcacgtgcatggcgcccagacttaatcgtcggtggtactatgagctatgtcgctccgctgttagctcttcacctgggagtcccgcacgcccgtcagacttgggatgcggtagacgctgatggaatccacccaggtgctgatgctgagcttcgcccagagttaagcgaattgggattggagcgccttcccgcacccgatttgttcatcgacatttgcccgccctcgttacgtcctgccaacgcagcaccagctcgcatgatgcgccacgtagccacgagccgccaatgcccgttagagccgtggatgtatacacgtgacactcgccagcgtgttttagtgacgtcgggatcgcgtgttgcaaaagaatcttacgatcgtaatttcgattttttacgtggattagcgaaggatttggtgcgctgggatgttgaattaattgtggctgctcctgacaccgtggctgaggctcttcgtgccgaggtgccacaagctcgcgtagggtggacccctttagacgtcgtggcccctacatgcgatttattggtgcatcacgccggcggagtctctacgctgactggtttatcggctggcgagccccaattattaatcccaaagggcagtgtattggaagctcctgcgcgccgcgtagcagattacggcgcggcgattgcactgttgcctggtgaggactcgacggaagctatcgccgatagttgtcaggagttgcacgccaaggacacttatgcccgccgcgctcaagacttaagccgcgaaatttcagggatgcctctgccggccacagtggtgactgcactggaacagttagcctaa

SEQ ID NO: 42 - DNA, 1548 bp, Unknown
  Dactylopius coccus
atggagttccgcttattgattctggcactgtttagtgtcttaatgagtacgtcaaatggtgccgagattcttgccctgtttccaattcacggaatttccaactacaacgtagcagaggcacttcttaaaacgcttgccaaccgtggacataacgtcactgtggtcacgtcattcccccagaagaaacccgtgccaaacttgtatgaaatcgacgtatctggggccaaaggtcttgctaccaactcaattcactttgagcgtcttcagactatcattcaagacgtgaagtccaacttcaagaatatggtgcgtctttcacgcacttactgcgagattatgttctccgatcctcgcgtacttaacatccgcgacaaaaagtttgatttggtaatcaacgcggtgttcggatcggattgtgacgctggctttgcgtggaaaagccaagcacccctgatctcaattttaaatgcacgccacaccccgtgggcgcttcaccgtatgggaaacccttctaaccctgcgtacatgccagtaatccactcacgcttcccagtaaaaatgaatttcttccagcgtatgatcaatacaggctggcatttatactttttgtatatgtacttttattatggcaacggagaagacgcaaataaaatggcgcgtaagtttttcggtaacgacatgcccgacattaacgaaatggtctttaacacatcgttgctttttgttaatactcactttagtgttgatatgccctaccctcttgttcctaactgcattgaaattggtgggattcacgtcaaagagccccaaccgcttcccctggagattcaaaaattcatggatgaagcagagcatggtgtaatctttttcactttgggctcgatggtccgcactagcacctttcccaatcagactatccaagcgtttaaagaggcgttcgcagaacttccacagcgtgttctttggaagtttgaaaacgagaatgaagacatgccttctaacgttttaatccgcaaatggtttccacagaacgatatctttggacataagaacattaaggcgtttatctcgcatggcggtaactcaggggcccttgaagccgtgcatttcggcgtgcccatcatcggcattcctctgttctatgatcagtatcgtaatatcttgagcttcgtgaaagaaggggttgcggtactgctggacgttaatgatttgacaaaggataacattctgtcgtctgttcgtacagtagtgaacgataaatcttacagcgaacgcatgaaagctctgtcccagctgtttcgcgatcgtccaatgagtcccctggacacggctgtctattggacggaatatgtaatccgtcaccgcggagcacatcatctgaagactgctggcgcttttttgcactggtatcagtatttgttgctggatgtgattactttccttttggtaacattctgtgccttttgcttcattgtcaagtacatctgtaaggcgctgattcaccattattggtcgagttccaagagtgaaaaattaaagaaaaactaa

SEQ ID NO: 43 - DNA, 1428 bp, Zea mays
atggctgctaatgggggggatcatacctccgcgcgcccacatgtggtgttgcttccatccgctggcatgggacatcttgtccctttcgcccgcttagctgtggctttatctgagggacacggctgcaacgtaagtgtagctgcagttcaaccaacggtttcctctgcggagtcgcgtctgttagacgcacttttcgtcgccgccgccccagccgtccgccgtcttgatttccgcctggcccccttcgatgaatccgagttccccggtgcagacccttttttcttacgcttcgaggcgacacgtcgctcggcaccgcttctggggccgttattagatgcggcggaagcctccgcacttgtgactgatattgtccttgcttcggtagcgttgccagtggcgcgcgagcgtggagttccctgctatgtgctttttacgtcatcggccgcaatgctgtcgttgtgtgcgtattttccagcttatttagatgcacatgcagcggccggctcggtcggggtcggagtagggaacgtcgacattccaggggtatttcgcatccctaagtcgagcgtcccgcaagcacttcacgatccagatcatttatttacccagcagtttgtcgcaaatggccgttgtttagttgcctgcgacggcattcttgttaacaccttcgacgccttcgagcccgatgcagtaaccgcactgcgccaagggtcgatcacagtctctggcggttttccaccagttttcaccgtgggcccaatgcttcccgttcgcttccaggcagaggagacggctgactacatgcgttggttgtctgcacaaccaccccgcagtgtcgtctatgtctcgtttggaagtcgcaaggcgattcctcgcgaccagttacgtgaattggccgcagggttagaggctagtggcaagcgttttctgtgggtagtaaagtcgaccatcgtcgaccgcgatgataccgccgatctgggcggcttgttgggggacggctttcttgagcgcgtccaaggtcgtgcatttgtgactatgggatgggtggaacaggaagagattttgcaacatggctcggttggcttgtttatctcgcattgtgggtggaatagccttaccgaagccgccgcgttcggggtaccagttcttgcctggcctcgtttcggagatcagcgtgtgaacgccgccttagttgcgcgctctggattgggagcgtgggaagaagggtggacttgggatggtgaggagggacttactacacgcaaggaagtggcgaaaaagatcaagggcatgatggggtacgatgctgtagccgaaaaggcggccaaagttggtgacgcagctgcggcagcaattgcaaaatgtggcacgagttatcaatctttggaagagtttgtacaacgttgccgcgacgccgagcgtaagtaa

SEQ ID NO: 44 - DNA, 1416 bp, Oryza sativa
atgccttcctcaggagacgctgccggtcgtcgccctcacgtcgtgctgatcccttcagccggaatggggcacctggtcccgtttggtcgtctggctgtcgcactttcctctgggcacggatgtgatgtgtctttagtaacagttcttcctactgtgagtacagcggagtcaaagcatcttgatgcactttttgacgcattccccgcagttcgccgtcttgacttcgagttggcgccatttgacgcatcagagtttcccggtgctgaccctttcttccttcgttttgaggcgatgcgccgttcggctccattgcttggccctttgctgacgggcgcgggcgctagcgcactggcgacggacattgctttaacgtctgtcgtaattccagtagcaaaagagcaagggcttccgtgtcacattttattcactgcgtcggccgcaatgttatcattgtgtgcctacttcccaacttatttggatgccaacgctggcggagggggcggtgtgggcgacgtggatattcctggagtgtatcgcattccgaaggcatcaattccacaagccttacatgatcccaaccacttgtttactcgtcagtttgtggcgaatggtcgtagtcttacctcggcggccggtattctggtgaacactttcgatgcgttagagccggaggcagtagctgcattgcagcaaggaaaggtagcctccggctttccaccagtattcgcggtggggccgttgctgcctgcctctaaccaggccaaggatccgcaggcaaattacatggagtggctggacgcccagcccgcccgcagcgtagtttatgtaagtttcgggagtcgcaaggcgatttcacgtgaacaacttcgcgagctggctgctggcttagaggggagcggccaccgttttctgtgggtcgtgaaatccaccgtcgtggatcgtgacgacgcggccgagctgggagagctgttggacgagggttttttagagcgtgtcgagaagcgtggattggtgacaaaggcatgggtcgaccaggaggaggtactgaaacatgaaagcgtagccctgtttgtctcacattgcggctggaacagcgtgactgaggcggcggcgagcggtgtgcctgtcctggccttaccccgcttcggggaccaacgtgttaattcaggagtggtggcacgtgcaggattaggagtatgggcggatacttggtcgtgggagggcgaagcaggcgtgattggtgcggaggaaatctcagagaaggtcaaagcagctatggccgacgaagctttacgtatgaaagctgcatcccttgcagaggcagccgccaaggcagtggctggcggtgggagtagtcatcgctgtttagcggaatttgcccgtctgtgtcaaggtggaacttgccgtactaattaa

SEQ ID NO: 45 - DNA, 1443 bp, Glycine max
atgagttctagtgaaggagtggtacatgtagcttttcttccaagtgcaggaatgggccacttgaaccctttccttcgcttggcggcgaccttcattcgttatggttgtaaagtaacgttaatcaccccgaagcctactgtatccctggcagaatcgaatttaatttcacgcttttgttccagctttccacatcaggttacgcaactggacctgaatttagtcagcgttgatccaacgaccgttgacacaatcgacccattcttcttacaatttgaaaccatccgccgtagtctgcatcttttacctcccattttaagtcttcttagcactcctttgtctgccttcatttatgacattactcttatcacgcctttgctttctgtaatcgagaagctgtcgtgccccagctacttgtattttacatcttcagcacgtatgttctctttcttcgcacgtgtctccgtgttgtccgcatctaatcccgggcagactccctcgtcatttatcggtgacgatggagttaagatccctgggttcacaagccccatcccacgcagcagtgttccgcctgcgattcttcaagcgtcctcaaatctttttcagcgcattatgttagaagacagcgcgaacgttaccaagcttaataatggggtcttcatcaatagctttgaagaactggagggcgaagctttagccgctttaaacggggggaaagttcttgaaggtctgccgcccgtgtacggggtgggcccccttatggcgtgtgaatatgagaaaggcgacgaggagggtcaaaagggctgcatgtcttcgatcgtgaagtggctggatgaacagtcgaagggaagcgtggtatacgtgtccttgggcaatcgtacggaaacgcgccgtgagcagattaaggatatggcccttggtttgatcgagtgtggctatggattcttgtgggtcgtcaaactgaagcgcgtcgataaagaagatgaggaaggcttagaagaggtgttaggtagcgagctgagttccaaggttaaggagaagggtgttgtagttaaggaatttgttgaccaagtcgaaattttgggccacccaagtgttgggggatttttgtcgcacgggggttggaacagcgtaactgaaactgtatggaagggagtgccttgtctgtcatggccacagcatagtgatcagaagatgtctgcggaggtaatccgtatgtccggaatgggtatctggcccgaggagtggggctgggggacgcaagatgttgtgaagggagacgaaatcgccaaacgcattaaggaaatgatgtcgaacgaatcgttgcgcgtaaaggcgggagaattgaaggaagcggcgttaaaggcggcaggggtaggggggagttgtgaagtgactattaaacgtcagatcgaagagtggaaacgcaatgcccaggctaattaa

SEQ ID NO: 46 - DNA, 1434 bp, Gentiana triflora
atggggagtttgactaacaacgataatcttcatatttttcttgtgtgcttcatcggccagggcgtggtcaatcccatgttacgtttggggaaggcgttcgcctccaaagggttacttgtcactttaagcgcaccggaaatcgttggaactgagatccgtaaggcgaataaccttaatgatgaccaaccaatcaaggtgggttccgggatgattcgtttcgaatttttcgacgatggatgggaatccgtaaacggtagcaaaccgtttgacgtatgggtctacatcaatcacttagaccagacaggccgtcaaaaacttccgattatgttaaagaaacatgaggagacagggactcctgtatcttgcttgatcctgaatcccttagtcccttgggtcgcggacgtagccgattcacttcagatcccctgcgctaccttgtgggtccaatcttgtgcaagtttttcagcatattaccactaccaccacgggttagtgcctttcccaaccgaatcagagcccgagatcgacgtacaacttcctgggatgccacttttgaaatatgatgaagtgcccgactacctgcatccgcgcacaccctaccccttttttggcacgaacattttaggtcaattcaagaatttatccaagaacttctgtatcctgatggataccttctacgagttggaacacgagatcatcgataatatgtgtaaattgtgtccgattaagccaattggcccgttgtttaagattccgaaagacccaagctccaacggaatcacgggtaatttcatgaaagtggatgactgcaaggagtggctggacagccgtccaacatcaactgtggtttacgttagtgtcgggtctgttgtatatttgaagcaggagcaggttacagaaatggcatacggcattttaaattcggaagtttcgtttttgtgggtgctgcgcccgccgagcaaacgcatcggtacggaaccgcatgtactgcccgaggagttctgggagaaggccggagatcgtggcaaggtggtgcaatggtcaccccaggagcaggtgcttgctcaccccgccactgtcggttttttaacacactgtggatggaatagcactcaagaggcgatttcgagcggagtgcccgtcatcactttcccacaatttggggaccaagtgaccaatgctaagttccttgtggaggaatttaaggtcggggtccgtttaggccgcggagagttagaaaatcgcatcatcacacgcgacgaagtagaacgcgctttacgcgagattacttcaggccccaaggctgaagaggtaaaagagaacgccttaaaatggaagaagaaggcagaagagacagtagctaaaggcggctactccgaacgtaatcttgtaggcttcattgaagaggtggctcgtaagactggtacaaagtaa

SEQ ID NO: 47 - DNA, 2112 bp, Aloe vera
atggaggaaatttccagtaaagtggagttcttatcccttaagcccagcatgtcaggaagtccccgttacagccccacatttcgtaaaatcggaagcggtcgcaattcccgccgcgactcccgtgctcatgcagggaatttcccctggattcgcaacaatcgtgtttttttttggctgcttttaatcaccatctgggcgtacatcggctttcacgtccaatctcaatgggcacatggcgaccataaagctgagttcgttggatacaagtcggaggtagggaagatgggtgaggacgtcaagtcggtaaatagtacgactacgttctccattgtacacaagggcaatttaactgttgaaggaaagaaagaccccgattccaattttggtatttcactgttgaaaaagggtaaacaggttctttcccgtttaaattcacgcaaaaagggccatcgttcgcgcaaggtgtcggaaaaactggaagaagaaacggacgacaatgggacgggagaaatggatgaggtccttatccagcgcaaaaacacatcttatggcttaattgtagggccttttgccaaactggaagagagtgtgcttgagtggagcccaggcaagcgccgtggtgtctgctatcgtaagggagaatttgcccgcgcggtgtcttctcagcgctttatgttgatcttccacgaattgtcaatgactggcgccccattgtccatgttggaattggccacggagatcctgtcttgcggtgggtctgtgagcgctattgtattatctaagaagggagggttaatgccggaactgaagaagcgtggtattaaggttttgcaagaccgtgacaaggtgagtttcaaggtcgccacgaaagtagacctgattattgcgggatctgctgtatgtagtagctggatcgagccatatctggagtatttccccgctgggtccggacatattgtctggtggatcatggaaaaccgtcgcgaatacttcgaccgtagcaagcatcttttaaaccgtgtgaaaattttggcatttcttagcgatagccagtcaaagcagtggctttcttggtgtgaggaagagaagattaaattcctgatccagccaatgttagtgccgttgtcagttaacgatgagctggccttcgttgccggtattccttgtagcttgaatactccagcattatcagtggagaaaatgatcgaaaagcgtgatttattacgtcacgcagtccgtaaggaaatggggttgggggacaatgacatgcttgtgatgagtttaagtagcatcaacccagccaagggtcagcgctttctgcttgaggcagccttactggtagctgaacacaatgtatcattgaaagatgctaacagttacagtcttatggaggaggagaagttatccgggaacgcacctcaaaatcaaaccatcatgatcggtcaactgaatcctggccacgtacttcagatcgccaatgacactaataagcccgtcaatgcgttacagaagattggcgccacacgtgtctcgtcgaagcgtcgcggcaagctgcatacgaatacagtcacgggcgtgcttcagaaaagccgcaaacttttgtccgaggcagcaggtatgaaggaggaaaccctgaaagtccttgtaggttccgtcggatcgaaatcgaataaggttctgtatgtaaaggcaatcatggaatacatcagccaacattctaatttgtctaaggtcgttctttggaccccagccaccacgtctatcgcagcactgtacgccgccgcggacgtgtacgtcattaacgctcagggacatggagagacattcggtcgcgtgacgatcgaggcgatggcctttggcctgccagtgctggggactgacgccggagggactaaagaaatcatcgaccaccgtgttacgggacttctgcatcctgtgggtcccgagggcactgtactgttagcgcaacacattcaatatcttttaaaaaatcccagcgtgcgcaagaaaatgggtatcaatggtcgccgcaaagtacaagataaatacttaaaacaccagacttacgagtcccttggcaaagtcatgttcaaatcgatgcgtccccgttaa

SEQ ID NO: 48 - DNA, 1611 bp, Unknown
  Streptomyces peucetius ATCC 29050
gtggccttgacgaagccggatgtcgatgtcctcgtggtgggcggcggtctcggggggctgtccaccgccctgttcctcgcccgccggggggcgcgggtcctgctggtggagcggcatgccagcacctcggtcctgcccaaggcggcaggccagaacccgcgcaccatggaactgttccgcttcggcggcgtggccgacgagatcctggccacggacgacatccgcggcgcccagggcgacttcaccatcaaggtcgtggagcgcgtgggcggtcgcgtcctgcacagcttcgcggagagcttcgaggaactggtcggtgcgacggaacagtgcacgcccatgccctgggcgctcgctccccaggaccgggtggagcccgtcctggtggcccacgccgccaagcacggcgcggagatccggttcgccaccgaactgacctccttccaggcgggcgacgacggtgtcacggcccgcctgcgcgacctgggcacgggagcggagagcaccgtgagcgcccgctacctggtcgccgccgacggaccccgcagcgcgatccgggagagcctgggcatcacccggcacggtcacggcaccctggcccacttcatgggcgtcatcttcgaggccgacctcaccgccgtcgtaccgcccgggtccaccggctggtactacctgcagcacccggacttcaccggcacgttcggccccaccgaccggcccaaccggcacaccttctacgtccgctacgaccccgaacgcggcgagaggccggaggactacacaccgcagcgctgcaccgagctgatccggctggctgtcgacgcgcccgggctcgtcccggacatcctcgacatccaggcctgggacatggcggcgtacatcgccgaccggtggcgcgaagggccggtgctgctggtcggcgatgccgccaaggtcaccccgcccaccgggggcatgggcggcaacaccgccatcggcgacgggttcgacgtggcctggaagctggccgccgtgctgcgcggcgaggcgggcgagcggctcctcgacagctacggggcggagcggtcgctcgtgtcccgcctcgtcgtcgacgagtcactcgccatctacgcccagcgcatggctccccacctgctcggcagcgttcccgaggaacgcggtacggcgcaggtcgtcctgggcttccgctaccgctccaccgccgtcgccgccgaggacgacgaccccgagccgaccgaggatccgcgacgcccgtccgggcgccccggcttccgcgcaccccacgtctggatcgaacaggacggcacacggcgttccaccgtcgagttgttcggcgactgctgggtgctcctggccgcaccggagggcggcgcctggggccaggcggccgcccgcgccgccgcggatctgggcgtccgcctcgacgtccatctcgtcggccgcgatgtcgccgccccctccggcgaactgacgcggacctacgggatcggccgggcgggggccagcttggtgcgcccggacggcgtggtcgcctggcgtacggcagtagcgccgggagcggaggcccaggaccagctgagcaccctgctcacccggctgctggcccgctga

SEQ ID NO: 49 - DNA, 2678 bp, Photorhabdus luminescens
atgataataaataacagaaatgaatctcaaccacgtagagttgtggtgacagggctaggtgttgtcgcaccgacaggtgttggcgttaatgaattttggaacaatattcataacggcaaatcgggggtaagtgaatatgagtggggaagaaaaaaatttggttttaaaagcggagcaataggaaaagttcacggtaacgatagcgatagcaaagagtttgtgctgaaaagtgagcgtaaatatcttgagtttgcgctagaagcctctgagatggcaatgcaagatgcaaatttaaaaccttcagacattgatggccggcgttttggcgttgcgatagcaacagcgattgccgatgctgcgggaatggaagagtgtttgctcaggatcaccaaagggggcaaagagaatattcatcctgatttaattaaatcagaggattatgacagctttgatttcagctctgccgccacctctgttgcgaaaaaatatggcgcatcgatgtccgtcagtaacatatcaactgggtgtgcggcaggacttgatgcattaggcattgcgatggagcatatccgttatggcagagcggatgtgatgctggctggcgccagtgaagcgccgctttgtccactttctatcggctcttttgaagctttaggggcgctatcatcaagagaattggaaaatcagcaagcagcgacttgtcctttttcccttgagcgggatggatttgtgattgctgaagggtgtggaatattaattttagagtcttatgaacatgctaagcagcgtggagcacatatctatgctgaattagcagggtatgcgtccgtgaataacgcttatcatatgaccgacttgcctgcggatggaatggcaatggcgcggtgcattgatatggcgttgaaggatgcccagatatcgccatcagcggtcaattatattagtgctcatggcagttctacggctcaaaatgatattaacgaatcaaatgcgattaaatttgttttgggagaaaatgcatttgatattccaattaactcattaaagtcaatgacaggtcatgctttagctgccgctaatgcgatcgagtctgtagcgttatgtctggaaatagaaaagcaatatattcatccaacaattaattatcaaacgccggaccctgattgcgatttagattatattcctaatcaaggttgcgcatatccaattaagaccgcattaaaattatcgagtggtttttctggtattcacagtgttattgttatgagggcagtagacaatgcgtaaaagagttgttgttaccggcgttggcgcagtacatcctgatggcaatgatgtcaccgctataaaaacaaaagtgattcagaaattattgggtcaggaatcgataaataataccaacaaaagttctgtaataaggacattgaatgatttcgatggggcaaaatatatcaataaccgcttaagacgtaaaattgatgaattttcagtttatggtatcgtcgccgttgaaatggcattaaaagcgagcagattggatgtagataagcttgatcctaatcgtgttggcatatatgttggaaactgttttggcggatggcagcatattgaggatgaagttaaagcgctccatgttgaaggcatatcggggatgggaccttatgttgctacggcatggttccctgctgcgcttcaagggcaattgtcactgctttatggttttagtgcgcaatctaagacattttccacctccgatgtagcagggatgcaagcaataggctatgcggctgaagcgatttctaatggtgttgccgaagtgatgttatgtggcgcgtcagaacatctttccagcccgttagttaaaagtttactggagaaagagtcaagccagaaacactctgaggtttttggcgaaagacagccaggggacttttccgaaggcgctgcatttctagtgctggaagagaggcaacatgctttagaacgcggcgcttcgatattgtgtgaattaacgggttttgttgattatttttcaccggataaaaatacaagaaataacaccttagaatatactgctgaactattcaaccataatgagaatgctgtatttattatggatggaatatatgatgatgaaaaagaaataacgagtaaggctttctccaataaagagataaaaacatcatttataaatctgaggccttacttgaataatcaattttcagtcagcggcgtaattgattcagtcctggcatcatcatttttatcagaaaataacggggatggagaacaacaatctaataaaataaatgaactttcaaatactaaccaaataataattcagcgctttagtaaccagggtcatgtatgtgcgttgagtttttcagcaatttaatctctaaaatatttaattacgcgaggaaaaatatatgaataataacccagaagtaaaaataaaaacgattttgtctctttttcttaacgttaatattgatgatttcaatatggatgcaaaccttgctgatgcctatgatatggattctacggaattggctgacttggcaaaagagattacgaaagagttcggtatttccgtgacgaaaagtcagttcagtcattgggaaacaggaagagccgttcttgatttcgtctcatcaagtttaaacgataaaaattaa

SEQ ID NO: 50 - DNA, 714 bp, Photorhabdus luminescens
atggacgatatttctttatcatctgatttttttgatctttggattatcaaaatcgacgatattgatttagcttctattgaacagttaattcactgttctgatatagttcgccataaccaaatttgtttagcggatagaagaaagagatttatatttagacgggctgcattacgttatgttttgagtcaatatttatctgattatgaaatcataacgaatgataacggaaaaccttatatatccacggagcaagacttcaaatattatttttcactgagtgcttcaggaaactattgtgccattggttttagctcaagggaaataggtgttgatattgaagtcactccttctaaggtaaaattttcagaaattattgaacgttttattaaggataaagatttggaatatatgaaaggtataatgttaaaacaactatcaggagttagtctcggatttaataactattatcatttaatgtcattatattattgggttagacttgaagcatatattaaattatttgcttcgactttacatgagaaattattggttaataactctgattctgttaaagatatgaaagaattggaggcaagcacattattgattcatagtcagcaatttgtttgtgccttatctcaaaagaaagtcatttctacaccaaatatcaaggaaataaattattccgaaattataaggaacaaagatgagtaa

SEQ ID NO: 51 - DNA, 1548 bp, Photorhabdus luminescens
atgaaactaatctctatgttgttacattcagagcatgataacttacatcatgattgtattgtcactaaggattatcattatacaagaaaagaggtgatatcttctgtttcccatttaattgatgatttattgagtcgaggagtgcaaaaaggtaataaagtcattgttatatttgaacatgatgaattaggtgttttctttttggctgccgccagtgctatggggttgcatttattaatgccctataatttatcatcagcgacaatcgatgaatggattaattttaccaatgaagtgcaatacgattttgttgtttatctcaaaaaagataaacattttgttggaaaattaaaagaaaacaacattaatgttattgatatttcagatcataagatcagagttagtgatgatattgcggaaatcccaatgataacttattctccgcaacctattgctaactttattgtcctgttcaccagtgggagtacaggcaaaccaaaagccattagtatttcagaatcgttagtatgtcgtcgaatttattcggtgaccgagaaattaaaatttacgcaagatgccaaaatattcatgtcaggtttgttgaataatacaactggagtgattttttctttcggctcattattgcatcaatcaacactttttatacccgaagatagaaatgtagagagatggcctgattatctttctcgcaataaaatcactcatattatgttacgcccagaatcaatgaaattattcgttaaatcgacagcagaacttaatattgatctctcttgtttacgggtggttgcttatggcgctgcggcgatgcctcctagcgtacttgagaaagggcgacaattaattggctgtgaatgggtgcagggatatgggttaagtgaaacttatggtcctttctgttgggtggatgagcaagatcatcgtgataaaagatatctcaattcaatttattgtgttggtaagattgataatacattggaagtggcagttaaacctattataggttcatcggataatatcggagaaattatactaaggggtaaaagtattatggaaggatattatgatgtcctttctggagaaataacgcctcctgatgaatggtttgccactggtgatcttggttatatagatgaagagggttatttagttttgaaaggacgtaagcaaaatacgtttatgagtgctaacggacacagaatttatcctgaagaaattgaatctattttatcccgaatacccaatgtgaatgtcgctacggttgttggtttttctttccatgaaaatggtgttgctattgatcagccggttgcttgcatgagtggagagatatctaagaagtcattacctgaaattgaagatattatttcatcatttttaatgagtaaactcagtcgagaaaaatggccggattggttctatgttactgatgaatgctttccgaaaagccataatgataagatattgaaatcagagttaattaaatcaatcgatcctaagaaattatttacattgaggaatcaataa

SEQ ID NO: 52 - DNA, 951 bp, Streptomyces coelicolor
atgctcgtactcgtcgctcccggccagggcgcccagacgcccggcttcctgactgactggctcgccctccccggtgccgctgaccgcgtcgccgcgtggtcggacgccatcggactcgatctcgcccacttcggcaccaaggccgacgcggacgagatccgagacacgtccgtggcccagccgctgctggtcgccgccggaatcctgtccgccgcggcactcggtacgcagacatctgtcgctgacgcgacgggccccgggttcacccccggcgcggtcgccggacacagcgtcggcgagatcaccgccgccgtcttcgcgggcgtcctcgacgacaccgccgcgctgtccctcgtacgccgtcgcggcctggccatggccgaggccgcggcggtcaccgagaccggcatgtcggcgctgctcgggggcgaccccgaggtgagcgtcgcgcacctggagcggctcggcctgaccccggcgaacgtgaacggcgccggtcagatcgtggcggcgggcaccatggagcagctggccgcgctgaacgaggacaagcccgagggtgtgcgcaaggtcgtcccgctgaaggtggccggcgcgttccacacccgccacatggcccccgccgtggacaagctcgccgaggccgccaaggcgctgacgccggccgacccgaaggtgacgtacgtctccaacaaggacgggcgggccgtcgcctccggcaccgaggtgctggaccggctggtcggccaggtcgccaacccggtgcgctgggacctgtgcatggagacgttcaaggagctgggcgtcaccgcgatcatcgaggtgtgtccgggcggcacgctgaccgggctggccaagcgggcgctgcccggagtgaagacgctggccctgaagacccccgacgacctcgacgcggcccgtgagctcgtcgccgagcacacccaggcctaa

SEQ ID NO: 53 - DNA, 1146 bp, Streptomyces coelicolor
atgagcgaggacacgatgacccaggagcggccgtccctgacggcacacgcccgccggatcgccgaactcgccgggaagcgggcggccgacgccgaacagcagcgccggctgagccccgacgtcgtcgacgcggtccttcgagccggtttcgccgcccacttcgtaccggtggcgcacggcggccgggccgcgacgttcggggagctggtggagcccgtcgcggtgctcggcgaggcctgtgcctcgaccgcctggtacgcctcgctcacggcgagcctcggccggatggccgcctacctgccggacgagggccaggccgagctgtggtccgacggccccgacgccctgatcgtcggtgccctgatgccgctgggccgggccgagaagaccccgggcggctggcacgtgtcgggcacctggccgttcgtcagcgtcgtggatcactccgactgggcgctgatctgcgccaaggtcggcgaggagccgtggttcttcgcggtgccgcgacaggagtacgggatcgtcgacagctggtacccgatgggtatgcgcggaacgggcagcaacacgctcgtcctcgacggggtgttcgtgccggatgcgcgggcctgcacccgtgcggccatcgcggcaggtctcggtccggatgccgaggcgatctgtcacaccgtgcccatgagggcggtcaacgggctggccttcgcactgccgatgctcggcgcggcccgcggggccgcggccgtgtggacctcgtggaccgccggaagactggccgggccgaccgggcagaacgccgtctcgtcccaggaccgcgtggtgtacgagcacacgctggcccgggccacgggtgagatcgacgcggcccagctgctgttggagcgggtcgcggcggtcgccgacgccggctcggcgaccggcgtactggtcggccgcggggcgcgggactgcgccctggcggcggagctgctgaccgccgcgaccgaccggctgttcgcctcggcgggcacccgggcacaggcccaggacagcccgatgcagcgcctgtggcgcgatgtgcacgcggcgggcagccatatcgggctgcagttcgggcccggggcggcgctgtacgccggagagctgttgaggaggagcaacgatggctga

SEQ ID NO: 54 - DNA, 534 bp, Streptomyces coelicolor
atggcagccgaccagggaatgctccgggacgccatggcccgggtgccggccggggtggcgctcgtcaccgcccatgaccgcgggggagtcccgcacggtttcaccgccagttcgttcgtgtccgtctcgatggagccgccactggcactggtctgcctggctcgtacggccaactccttcccggtgttcgacagttgcggcgagttcgcggtgagcgtgctgcgcgaggaccacacggacctggccatgcgcttcgcgcgcaagtccgcggacaagttcgcgggcggggagttcgtccgtaccgcgcggggagcgaccgtgctcgacggagcggtcgcggtcgtcgagtgcacggtccacgagcgctacccggcgggcgaccacatcatcctgctcggcgaggtccagtccgtgcacgtcgaggagaagggcgtaccggcggtctacgtggaccgccggttcgccgccctgtgctcggcggcgggtgcctgcccgtccgccaccgggcggggcgtgcccgcgcatgccggctaa

SEQ ID NO: 55 - DNA, 1194 bp, Pseudomonas fluorescens
atgaaaacgctaaaaacccaagtcgccattattggcgccggtccctccggattgctgctcggccagttactgcacaacgcgggtatccagaccctgattctagagcgccagagcgccgactacgtgcaaggccgcatccgtgccggggtgctggagcaaggcatggtcgacctgctgcgcgaagcgggcgtcagccgacgcatggacgccgagggccttgtgcatgacggtttcgaattggcactcaatggcgaactcacccacatcgacctcaaggcgctcaccggcggccagtcggtgatgatctacggccagaccgaagtcacccgtgacttgatggccgcccgcgaagcggcgggtggcatcactctatacgaaacgcagaacgtgcagcctcatggtcacaaaactgatcgaccctggctgaccttcgagcaccagggtgaagcttttcgcctggagtgcgactacatcgcgggctgtgatggttttcacggtgtggcgcggcagtcgattccggcgcagtcgttgaaggtcttcgagcgcgtctatcccttcggttggctgggcgtcctcgccgacacaccgccggtgcatgacgaactggtgtacgccaaacatgcgcgtggctttgccctgtgcagcatgcgctcgccgacccgcagccgctattacctgcaagtgccggttgaagaagcgctggatgaatggtcggatcagcgcttctgggatgagctgaaaacccgtttgcccagtgcactggcggcccaactggtcaccgggccatccatcgagaagagcatcgcgccgctgcgcagctttgtggtcgagccgatgcaatacgggcgcctgttcctgctgggggacgccgcgcatatcgtgccgcccaccggggccaagggcttgaacctggcggccagcgacgtgagtacgctgtttcggatcttgctcaaggtctatcgcgaggggcgggtggacctgctggaacagtactcagcgatctgcttgcgccgcgtatggaaagccgaacggttttcctggtggatgacttcgatgttgcaccagtttccggaggccgacgggttcagccagcgcattgccgagagcgagcttgcgtatttcatcagctccgaggcgggccgcaaaaccatcgcagaaaattacgtcgggcttccttacgaagctatcgaataa

SEQ ID NO: 56 - DNA, 1611 bp, Artificial Sequence
  dnrF P217K from Streptomyces peucetius
gtggccttgacgaagccggatgtcgatgtcctcgtggtgggcggcggtctcggggggctgtccaccgccctgttcctcgcccgccggggggcgcgggtcctgctggtggagcggcatgccagcacctcggtcctgcccaaggcggcaggccagaacccgcgcaccatggaactgttccgcttcggcggcgtggccgacgagatcctggccacggacgacatccgcggcgcccagggcgacttcaccatcaaggtcgtggagcgcgtgggcggtcgcgtcctgcacagcttcgcggagagcttcgaggaactggtcggtgcgacggaacagtgcacgcccatgccctgggcgctcgctccccaggaccgggtggagcccgtcctggtggcccacgccgccaagcacggcgcggagatccggttcgccaccgaactgacctccttccaggcgggcgacgacggtgtcacggcccgcctgcgcgacctgggcacgggagcggagagcaccgtgagcgcccgctacctggtcgccgccgacggaccccgcagcgcgatccgggagagcctgggcatcacccggcacggtcacggcaccctggcccacttcatgggcgtcatcttcgaggccgacctcaccgccgtcgtaccgaaggggtccaccggctggtactacctgcagcacccggacttcaccggcacgttcggccccaccgaccggcccaaccggcacaccttctacgtccgctacgaccccgaacgcggcgagaggccggaggactacacaccgcagcgctgcaccgagctgatccggctggctgtcgacgcgcccgggctcgtcccggacatcctcgacatccaggcctgggacatggcggcgtacatcgccgaccggtggcgcgaagggccggtgctgctggtcggcgatgccgccaaggtcaccccgcccaccgggggcatgggcggcaacaccgccatcggcgacgggttcgacgtggcctggaagctggccgccgtgctgcgcggcgaggcgggcgagcggctcctcgacagctacggggcggagcggtcgctcgtgtcccgcctcgtcgtcgacgagtcactcgccatctacgcccagcgcatggctccccacctgctcggcagcgttcccgaggaacgcggtacggcgcaggtcgtcctgggcttccgctaccgctccaccgccgtcgccgccgaggacgacgaccccgagccgaccgaggatccgcgacgcccgtccgggcgccccggcttccgcgcaccccacgtctggatcgaacaggacggcacacggcgttccaccgtcgagttgttcggcgactgctgggtgctcctggccgcaccggagggcggcgcctggggccaggcggccgcccgcgccgccgcggatctgggcgtccgcctcgacgtccatctcgtcggccgcgatgtcgccgccccctccggcgaactgacgcggacctacgggatcggccgggcgggggccagcttggtgcgcccggacggcgtggtcgcctggcgtacggcagtagcgccgggagcggaggcccaggaccagctgagcaccctgctcacccggctgctggcccgctga

SEQ ID NO: 57 - DNA, 1434 bp, Artificial Sequence
  GtCGT V93Q/Y193F from Gentiana triflora
atggggagtttgactaacaacgataatcttcatatttttcttgtgtgcttcatcggccagggcgtggtcaatcccatgttacgtttggggaaggcgttcgcctccaaagggttacttgtcactttaagcgcaccggaaatcgttggaactgagatccgtaaggcgaataaccttaatgatgaccaaccaatcaaggtgggttccgggatgattcgtttcgaatttttcgacgatggatgggaatccgtaaacggtagcaaaccgtttgacgtatggcaatacatcaatcacttagaccagacaggccgtcaaaaacttccgattatgttaaagaaacatgaggagacagggactcctgtatcttgcttgatcctgaatcccttagtcccttgggtcgcggacgtagccgattcacttcagatcccctgcgctaccttgtgggtccaatcttgtgcaagtttttcagcatattaccactaccaccacgggttagtgcctttcccaaccgaatcagagcccgagatcgacgtacaacttcctgggatgccacttttgaaatatgatgaagtgcccgacttcctgcatccgcgcacaccctaccccttttttggcacgaacattttaggtcaattcaagaatttatccaagaacttctgtatcctgatggataccttctacgagttggaacacgagatcatcgataatatgtgtaaattgtgtccgattaagccaattggcccgttgtttaagattccgaaagacccaagctccaacggaatcacgggtaatttcatgaaagtggatgactgcaaggagtggctggacagccgtccaacatcaactgtggtttacgttagtgtcgggtctgttgtatatttgaagcaggagcaggttacagaaatggcatacggcattttaaattcggaagtttcgtttttgtgggtgctgcgcccgccgagcaaacgcatcggtacggaaccgcatgtactgcccgaggagttctgggagaaggccggagatcgtggcaaggtggtgcaatggtcaccccaggagcaggtgcttgctcaccccgccactgtcggttttttaacacactgtggatggaatagcactcaagaggcgatttcgagcggagtgcccgtcatcactttcccacaatttggggaccaagtgaccaatgctaagttccttgtggaggaatttaaggtcggggtccgtttaggccgcggagagttagaaaatcgcatcatcacacgcgacgaagtagaacgcgctttacgcgagattacttcaggccccaaggctgaagaggtaaaagagaacgccttaaaatggaagaagaaggcagaagagacagtagctaaaggcggctactccgaacgtaatcttgtaggcttcattgaagaggtggctcgtaagactggtacaaagtaa

SEQ ID NO: 58 - DNA, 1176 bp, Unknown
  Rheum palmatum
atggcagatgtcctgcaggagatccgcaactcgcagaaggcgagcgggcccgccacggtgctcgccatcggcactgcccatccaccgacgtgctaccctcaggccgactaccccgacttctacttccgagtttgcaagagcgagcacatgaccaaactcaagaagaaaatgcaattcatttgtgacagatcggggataaggcagcggtttatgttccacacggaagagaacctggggaagaacccggggatgtgcacattcgacgggccatcgctgaacgcgcggcaggacatgctgatcatggaagtgccgaagctgggggcggaggcggcggagaaggcgatcaaggagtgggggcaggacaagtcccggatcacccacctcatcttctgcaccaccacgagcaacgacatgcccggggcggactaccagttcgccaccctgttcgggctgaaccccggcgtgagccgcaccatggtctaccagcagggctgcttcgccgggggcaccgtgctgcgcctggtcaaggacatcgcggagaacaacaagggggcgcgcgtgctggtggtgtgctcggagatcgtggccttcgccttccgcgggccccacgaggaccacatcgactccctcatcgggcagctcctgttcggggacggggccgccgccctcgtggtcgggacagacatcgacgagagcgtcgagaggcccatcttccagatcatgtcggcgacccaggcgaccatccccaactcgctgcacaccatggctctccatctgacggaggcggggctgaccttccatctcagcaaggaggtgcccaaggtggtgagcgacaacatggaggagctcatgctcgaggccttcaagccgctcgggataaccgattggaactccatattctggcaagtgcatcccgggggtagagccatccttgacaagatcgaggagaagctggagctcaccaaggataagatgcgggattcccgctacatcttgagcgagtacgggaatctcaccagcgcctgtgtgctctttgtcatggacgagatgaggaagaggtccttccgggaagggaagcagaccaccggagacggctacgagtggggtgtcgccatcggattggggcccggtcttaccgtcgagaccgttgtcttgcgtagcgtccccattccctaa

SEQ ID NO: 59 - DNA, 1776 bp, Unknown
  Corynebacterium glutamicum
gtgtcagtcgagactaggaagatcaccaaggttcttgtcgctaaccgtggtgagattgcaatccgcgtgttccgtgcagctcgagatgaaggcatcggatctgtcgccgtctacgcagagccagatgcagatgcaccattcgtgtcatatgcagacgaggcttttgccctcggtggccaaacatccgctgagtcctaccttgtcattgacaagatcatcgatgcggcccgcaagtccggcgccgacgccatccaccccggctacggcttcctcgcagaaaacgctgacttcgcagaagcagtcatcaacgaaggcctgatctggattggaccttcacctgagtccatccgctccctcggcgacaaggtcaccgctcgccacatcgcagataccgccaaggctccaatggctcctggcaccaaggaaccagtaaaagacgcagcagaagttgtggctttcgctgaagaattcggtctcccaatcgccatcaaggcagctttcggtggcggcggacgtggcatgaaggttgcctacaagatggaagaagtcgctgacctcttcgagtccgcaacccgtgaagcaaccgcagcgttcggccgcggcgagtgcttcgtggagcgctacctggacaaggcacgccacgttgaggctcaggtcatcgccgataagcacggcaacgttgttgtcgccggaacccgtgactgctccctgcagcgccgtttccagaagctcgtcgaagaagcaccagcaccattcctcaccgatgaccagcgcgagcgtctccactcctccgcgaaggctatctgtaaggaagctggctactacggtgcaggcaccgttgagtacctcgttggctccgacggcctgatctccttcctcgaggtcaacacccgcctccaggtggaacacccagtcaccgaagagaccaccggcatcgacctggtccgcgaaatgttccgcatcgcagaaggccacgagctctccatcaaggaagatccagctccacgcggccacgcattcgagttccgcatcaacggcgaagacgctggctccaacttcatgcctgcaccaggcaagatcaccagctaccgcgagccacagggcccaggcgtccgcatggactccggtgtcgttgaaggttccgaaatctccggacagttcgactccatgctggcaaagctgatcgtttggggcgacacccgcgagcaggctctccagcgctcccgccgtgcacttgcagagtacgttgtcgagggcatgccaaccgttatcccattccaccagcacatcgtggaaaacccagcattcgtgggcaacgacgaaggcttcgagatctacaccaagtggatcgaagaggtttgggataacccaatcgcaccttacgttgacgcttccgagctcgacgaagatgaggacaagaccccagcacagaaggttgttgtggagatcaacggccgtcgcgttgaggttgcactcccaggcgatctggcactcggtggcaccgctggtcctaagaagaaggccaagaagcgtcgcgcaggtggtgcaaaggctggcgtatccggcgatgcagtggcagctccaatgcagggcactgtcatcaaggtcaacgtcgaagaaggcgctgaagtcaacgaaggcgacaccgttgttgtcctcgaggctatgaagatggaaaaccctgtgaaggctcataagtccggaaccgtaaccggccttactgtcgctgcaggcgagggtgtcaacaagggcgttgttctcctcgagatcaagtaa

SEQ ID NO: 60 - DNA, 1321 bp, Corynebacterium glutamicum; identical to SEQ ID NO: 38

SEQ ID NO: 61 - protein, 477 aa, Artificial Sequence
  GtCGT V93Q/Y193F (GtUF6CGT1V93Q/Y193F) variant
MGSLTNNDNLHIFLVCFIGQGVVNPMLRLGKAFASKGLLVTLSAPEIVGTEIRKANNLNDDQPIKVGSGMIRFEFFDDGWESVNGSKPFDVWQYINHLDQTGRQKLPIMLKKHEETGTPVSCLILNPLVPWVADVADSLQIPCATLWVQSCASFSAYYHYHHGLVPFPTESEPEIDVQLPGMPLLKYDEVPDFLHPRTPYPFFGTNILGQFKNLSKNFCILMDTFYELEHEIIDNMCKLCPIKPIGPLFKIPKDPSSNGITGNFMKVDDCKEWLDSRPTSTVVYVSVGSVVYLKQEQVTEMAYGILNSEVSFLWVLRPPSKRIGTEPHVLPEEFWEKAGDRGKVVQWSPQEQVLAHPATVGFLTHCGWNSTQEAISSGVPVITFPQFGDQVTNAKFLVEEFKVGVRLGRGELENRIITRDEVERALREITSGPKAEEVKENALKWKKKAEETVAKGGYSERNLVGFIEEVARKTGTK

SEQ ID NO: 62 - DNA, 1321 bp, Artificial Sequence; identical to SEQ ID NO: 38
  zhuIJ - Codon optimization for E. coli

SEQ ID NO: 63 - DNA, 29 bp, Artificial Sequence
  GtCGT V93Q/Y193F_I18P_F
tgtgcttcccaggccagggcgtggtcaat

SEQ ID NO: 64 - DNA, 31 bp, Artificial Sequence
  GtCGT V93Q/Y193F_I18P_R
cgccctggcctgggaagcacacaagaaaaat

SEQ ID NO: 65 - DNA, 29 bp, Artificial Sequence
  GtCGT V93Q/Y193F_Q20M_F
ttcatcggcatgggcgtggtcaatcccat

SEQ ID NO: 66 - DNA, 31 bp, Artificial Sequence
  GtCGT V93Q/Y193F_Q20M_R
tgaccacgcccatgccgatgaagcacacaag

SEQ ID NO: 67 - DNA, 30 bp, Artificial Sequence
  GtCGT V93Q/Y193F_T50K_F
aatcgttggaaaggagatccgtaaggcgaa

SEQ ID NO: 68 - DNA, 30 bp, Artificial Sequence
  GtCGT V93Q/Y193F_T50K_R
tacggatctcctttccaacgatttccggtg

SEQ ID NO: 69 - DNA, 30 bp, Artificial Sequence
  GtCGT V93Q/Y193F_T50N_F
aatcgttggaaatgagatccgtaaggcgaa

SEQ ID NO: 70 - DNA, 30 bp, Artificial Sequence
  GtCGT V93Q/Y193F_T50Q_F
tacggatctcatttccaacgatttccggtg

SEQ ID NO: 71 - DNA, 30 bp, Artificial Sequence
  GtCGT V93Q/Y193F_T50Q_R
aatcgttggacaggagatccgtaaggcgaa

SEQ ID NO: 72 - DNA, 30 bp, Artificial Sequence
  GtCGT V93Q/Y193F_T50R_F
tacggatctcctgtccaacgatttccggtg

SEQ ID NO: 73 - DNA, 30 bp, Artificial Sequence
  GtCGT V93Q/Y193F_T50R_R
aatcgttggacgtgagatccgtaaggcgaa

SEQ ID NO: 74 - DNA, 30 bp, Artificial Sequence
  GtCGT V93Q/Y193F_T50V_F
tacggatctcacgtccaacgatttccggtg

SEQ ID NO: 75 - DNA, 30 bp, Artificial Sequence
  GtCGT V93Q/Y193F_T50V_R
aatcgttggagttgagatccgtaaggcgaa

SEQ ID NO: 76 - DNA, 30 bp, Artificial Sequence
  GtCGT V93Q/Y193F_T50V_R
tacggatctcaactccaacgatttccggtg

SEQ ID NO: 77 - DNA, 34 bp, Artificial Sequence
  GtCGT V93Q/Y193F_I95L_F
gtatggcaatacctcaatcacttagaccagacag

SEQ ID NO: 78 - DNA, 36 bp, Artificial Sequence
  GtCGT V93Q/Y193F_I95L_R
ggtctaagtgattgaggtattgccatacgtcaaacg

SEQ ID NO: 79 - DNA, 34 bp, Artificial Sequence
  GtCGT V93Q/Y193F_I95M_F
gtatggcaatacatgaatcacttagaccagacag

SEQ ID NO: 80 - DNA, 36 bp, Artificial Sequence
  GtCGT V93Q/Y193F_I95M_R
ggtctaagtgattcatgtattgccatacgtcaaacg

SEQ ID NO: 81 - DNA, 34 bp, Artificial Sequence
  GtCGT V93Q/Y193F_I95T_F
gtatggcaatacactaatcacttagaccagacag

SEQ ID NO: 82 - DNA, 36 bp, Artificial Sequence
  GtCGT V93Q/Y193F_I95T_R
ggtctaagtgattagtgtattgccatacgtcaaacg

SEQ ID NO: 83 - DNA, 32 bp, Artificial Sequence
  GtCGT V93Q/Y193F_V290A_F
gtgtcgggtctgctgtatatttgaagcaggag

SEQ ID NO: 84 - DNA, 32 bp, Artificial Sequence
  GtCGT V93Q/Y193F_V290A_R
gcttcaaatatacagcagacccgacactaacg

SEQ ID NO: 85 - DNA, 32 bp, Artificial Sequence
  GtCGT V93Q/Y193F_V290G_F
gtgtcgggtctggtgtatatttgaagcaggag

SEQ ID NO: 86 - DNA, 32 bp, Artificial Sequence
  GtCGT V93Q/Y193F_V290G_R
gcttcaaatatacaccagacccgacactaacg

SEQ ID NO: 87 - DNA, 29 bp, Artificial Sequence
  GtCGT V93Q/Y193F_I323A_F
agcaaacgcgccggtacggaaccgcatgt

SEQ ID NO: 88 - DNA, 25 bp, Artificial Sequence
  GtCGT V93Q/Y193F_I323A_R
gttccgtaccggcgcgtttgctcgg

SEQ ID NO: 89 - DNA, 29 bp, Artificial Sequence
  GtCGT V93Q/Y193F_I323S_F
agcaaacgcagcggtacggaaccgcatgt

SEQ ID NO: 90 - DNA, 25 bp, Artificial Sequence
  GtCGT V93Q/Y193F_I323S_R
gttccgtaccgctgcgtttgctcgg

SEQ ID NO: 91 - DNA, 30 bp, Artificial Sequence
  V22A-f
cggccagggcgcggtcaatcccatgttacg

SEQ ID NO: 92 - DNA, 30 bp, Artificial Sequence
  V22A-R
tgggattgaccgcgccctggccgatgaagc

SEQ ID NO: 93 - DNA, 30 bp, Artificial Sequence
  L29A-F
catgttacgtgcggggaaggcgttcgcctc

SEQ ID NO: 94 - DNA, 30 bp, Artificial Sequence
  L29A-R
cgccttccccgcacgtaacatgggattgac

SEQ ID NO: 95 - DNA, 30 bp, Artificial Sequence
  E46G-f
agcgcaccgggcatcgttggaactgagatc

SEQ ID NO: 96 - DNA, 30 bp, Artificial Sequence
  E46G-R
tccaacgatgcccggtgcgcttaaagtgac

SEQ ID NO: 97 - DNA, 30 bp, Artificial Sequence
  V48G-f
ccggaaatcggtggaactgagatccgtaag

SEQ ID NO: 98 - DNA, 30 bp, Artificial Sequence
  V48G-R
ctcagttccaccgatttccggtgcgcttaa

SEQ ID NO: 99 - DNA, 31 bp, Artificial Sequence
  E51C-f
cgttggaacttgcatccgtaaggcgaataac

SEQ ID NO: 100 - DNA, 31 bp, Artificial Sequence
  E51C-R
ccttacggatgcaagttccaacgatttccgg

SEQ ID NO: 101 - DNA, 35 bp, Artificial Sequence
  A55S-f
gatccgtaagtcgaataaccttaatgatgaccaac

SEQ ID NO: 102 - DNA, 30 bp, Artificial Sequence
  A55S-r
aaggttattcgacttacggatctcagttcc

SEQ ID NO: 103 - DNA, 31 bp, Artificial Sequence
  S86V-F
cgtaaacggtgtcaaaccgtttgacgtatgg

SEQ ID NO: 104 - DNA, 31 bp, Artificial Sequence
  S86V-r
caaacggtttgacaccgtttacggattccca

SEQ ID NO: 105 - DNA, 32 bp, Artificial Sequence
  D99G-F
caatcacttaggccagacaggccgtcaaaaac

SEQ ID NO: 106 - DNA, 32 bp, Artificial Sequence
  D99G-r
ggcctgtctggcctaagtgattgatgtattgc

SEQ ID NO: 107 - DNA, 31 bp, Artificial Sequence
  R103V-F
ccagacaggcgttcaaaaacttccgattatg

SEQ ID NO: 108 - DNA, 32 bp, Artificial Sequence
  R103V-R
ggaagtttttgaacgcctgtctggtctaagtg

SEQ ID NO: 109 - DNA, 31 bp, Artificial Sequence
  C151G-F
ggtccaatctggtgcaagtttttcagcatat

SEQ ID NO: 110 - DNA, 31 bp, Artificial Sequence
  C151G-r
gaaaaacttgcaccagattggacccacaagg

SEQ ID NO: 111 - DNA, 32 bp, Artificial Sequence
  L184G-F
ctgggatgccaggtttgaaatatgatgaagtg

SEQ ID NO: 112 - DNA, 31 bp, Artificial Sequence
  L184G-r
catatttcaaacctggcatcccaggaagttg

SEQ ID NO: 113 - DNA, 30 bp, Artificial Sequence
  L194A-F
cccgacttcgcgcatccgcgcacaccctac

SEQ ID NO: 114 - DNA, 32 bp, Artificial Sequence
  L194A-r
gtgcgcggatgcgcgaagtcgggcacttcatc

SEQ ID NO: 115 - DNA, 31 bp, Artificial Sequence
  E332P-F
tgtactgcccccggagttctgggagaaggcc

SEQ ID NO: 116 - DNA, 31 bp, Artificial Sequence
  E332P-r
cccagaactccgggggcagtacatgcggttc

SEQ ID NO: 117 - DNA, 31 bp, Artificial Sequence
  I18A-F
tgtgtgcttcgccggccagggcgtggtcaat

SEQ ID NO: 118 - DNA, 31 bp, Artificial Sequence
  I18A-r
cgccctggccggcgaagcacacaagaaaaat

SEQ ID NO: 119 - DNA, 31 bp, Artificial Sequence
  P385A-F
catcactttcgcacaatttggggaccaagtg

SEQ ID NO: 120 - DNA, 31 bp, Artificial Sequence
  P385A-r
ccccaaattgtgcgaaagtgatgacgggcac

SEQ ID NO: 121 - DNA, 43 bp, Artificial Sequence
  GtCGT_N_His_IV_F
caccatcaccatcaccatgggagtttgactaacaacgataatc

SEQ ID NO: 122 - DNA, 24 bp, Artificial Sequence
  GtCGT_N_His_IV_R
catatgtatatctccttcttatac